European Patent Application EP 4 285 926 A1, published December 6, 2023. Title: COMBINATION TREATMENT FOR CHRONIC LYMPHOCYTIC LEUKEMIA. Applicant: LAVA Therapeutics. The sequence listing filed with the application follows.

SEQUENCE LISTING (10 sequences)

SEQ ID NO: 1 - protein, 5 aa, Artificial Sequence
  antibody sequence
DNVMG

SEQ ID NO: 2 - protein, 16 aa, Artificial Sequence
  antibody sequence
TIRTGGSTNYADSVKG

SEQ ID NO: 3 - protein, 11 aa, Artificial Sequence
  antibody sequence
TIPVPSTPYDY

SEQ ID NO: 4 - protein, 119 aa, Artificial Sequence
  antibody sequence
QVQLVESGGGLVQAGGSLRLSCAASGSMFSDNVMGWYRQAPGKQRELVATIRTGGSTNYADSVKGRFTISRDNAKNTVYLQMNSLKPEDTAVYYCRHTIPVPSTPYDYWGQGTQVTVSS

SEQ ID NO: 5 - protein, 5 aa, Artificial Sequence
  antibody sequence
  VARIANT (5)..(5): X is G or S
NYAMX

SEQ ID NO: 6 - protein, 17 aa, Artificial Sequence
  antibody sequence
AISWSGGSTSYADSVKG

SEQ ID NO: 7 - protein, 21 aa, Artificial Sequence
  antibody sequence
  VARIANT (7)..(7): X is Y, F or S
QFSGADXGFGRLGIRGYEYDY

SEQ ID NO: 8 - protein, 130 aa, Artificial Sequence
  antibody sequence
  VARIANT (35)..(35): X is G or S
  VARIANT (105)..(105): X is Y, F or S
EVQLVESGGGLVQAGGSLRLSCAASGRPFSNYAMXWFRQAPGKEREFVAAISWSGGSTSYADSVKGRFTISRDNAKNTVYLQMNSPKPEDTAIYYCAAQFSGADXGFGRLGIRGYEYDYWGQGTQVTVSS

SEQ ID NO: 9 - protein, 254 aa, Artificial Sequence
  antibody sequence
EVQLVESGGGLVQAGGSLRLSCAASGSMFSDNVMGWYRQAPGKQRELVATIRTGGSTNYADSVKGRFTISRDNAKNTVYLQMNSLKPEDTAVYYCRHTIPVPSTPYDYWGQGTQVTVSSGGGGSEVQLLESGGGSVQPGGSLRLSCAASGRPFSNYAMSWFRQAPGKEREFVSAISWSGGSTSYADSVKGRFTISRDNSKNTLYLQMNSLRAEDTAVYYCAAQFSGADYGFGRLGIRGYEYDYWGQGTQVTVSS

SEQ ID NO: 10 - protein, 335 aa, Homo sapiens
MGCLLFLLLWALLQAWGSAEVPQRLFPLRCLQISSFANSSWTRTDGLAWLGELQTHSWSNDSDTVRSLKPWSQGTFSDQQWETLQHIFRVYRSSFTRDVKEFAKMLRLSYPLELQVSAGCEVHPGNASNNFFHVAFQGKDILSFQGTSWEPTQEAPLWVNLAIQVLNQDKWTRETVQWLLNGTCPQFVSGLLESGKSELKKQVKPKAWLSRGPSPGPGRLLLVCHVSGFYPKPVWVKWMRGEQEQQGTQPGDILPNADETWYLRATLDVVAGEAAGLSCRVKHSSLEGQDIVLYWGGSYTSMGLIALAVLACLLFLLIVGFTSRFKRQTSYQGVL